European Patent Specification EP 3 801 583 B1, published July 2, 2025. Title: RECOMBINANT HERPES SIMPLEX VIRUS FOR CANCER IMMUNOTHERAPY. Applicant: THE BOARD OF TRUSTEES OF THE  UNIVERSITY OF ILLINOIS He, Bin Liu, Xing. The sequence listing filed with the application follows.

SEQUENCE LISTING (22 sequences)

SEQ ID NO: 1 - protein, 248 aa, herpes simplex virus 1
MARRRRHRGPRRPRPPGPTGAVPTAQSQVTSTPNSEPAVRSAPAAAPPPPPASGPPPSCSLLLRQWLHVPESASDDDDDDDWPDSPPPEPAPEARPTAAAPRPRSPPPGAGPGGGANPSHPPSRPFRLPPRLALRLRVTAEHLARLRLRRAGGEGAPEPPATPATPATPATPATPARVRFSPHVRVRHLVVWASAARLARRGSWARERADRARFRRRVAEAEAVIGPCLGPEARARALARGAGPANSV

SEQ ID NO: 2 - protein, 102 aa, Artificial sequence
  Synthetic polypeptide
RLRRAGGEGAPEPPATPATPATPATPATPARVRFSPHVRVRHLVVWASAARLARRGSWARERADRARFRRRVAEAEAVIGPCLGPEARARALARGAGPANSV

SEQ ID NO: 3 - DNA, 26 bp, Artificial sequence
  Synthetic oligonucleotide
gccttgacactcctggtacaaatgag

SEQ ID NO: 4 - DNA, 24 bp, Artificial sequence
  Synthetic oligonucleotide
cagcacattggcagaggaagacag

SEQ ID NO: 5 - DNA, 20 bp, Artificial sequence
  Synthetic oligonucleotide
caaggcaggtttctgaggag

SEQ ID NO: 6 - DNA, 21 bp, Artificial sequence
  Synthetic oligonucleotide
aagcagattctccatgacctg

SEQ ID NO: 7 - DNA, 20 bp, Artificial sequence
  Synthetic oligonucleotide
ctgctgctttgcctacctct

SEQ ID NO: 8 - DNA, 20 bp, Artificial sequence
  Synthetic oligonucleotide
cacttcttctctgggttggc

SEQ ID NO: 9 - DNA, 23 bp, Artificial sequence
  Synthetic oligonucleotide
tccttccttccttccttccttcc

SEQ ID NO: 10 - DNA, 23 bp, Artificial sequence
  Synthetic oligonucleotide
aggctctttttcaccctgtctgg

SEQ ID NO: 11 - DNA, 22 bp, Artificial sequence
  Synthetic oligonucleotide
ggccttgacctttgctttactg

SEQ ID NO: 12 - DNA, 21 bp, Artificial sequence
  Synthetic oligonucleotide
cacagagcagcttgacttgca

SEQ ID NO: 13 - DNA, 20 bp, Artificial sequence
  Synthetic oligonucleotide
cctccttgggttcgtctaca

SEQ ID NO: 14 - DNA, 20 bp, Artificial sequence
  Synthetic oligonucleotide
agtggctgatatctgggtgc

SEQ ID NO: 15 - DNA, 20 bp, Artificial sequence
  Synthetic oligonucleotide
cctgctgctttgcctacatt

SEQ ID NO: 16 - DNA, 20 bp, Artificial sequence
  Synthetic oligonucleotide
acacacttggcggttctttc

SEQ ID NO: 17 - DNA, 23 bp, Artificial sequence
  Synthetic oligonucleotide
ccctgtttcttccacagtgccta

SEQ ID NO: 18 - DNA, 23 bp, Artificial sequence
  Synthetic oligonucleotide
gagacaatggtctggttgccatc

SEQ ID NO: 19 - DNA, 20 bp, Artificial sequence
  Synthetic oligonucleotide
cctgcggcttaatttgactc

SEQ ID NO: 20 - DNA, 20 bp, Artificial sequence
  Synthetic oligonucleotide
aaccagacaaatcgctccac

SEQ ID NO: 21 - DNA, 20 bp, Artificial sequence
  Synthetic oligonucleotide
tacaacctgaccatcgcttg

SEQ ID NO: 22 - DNA, 20 bp, Artificial sequence
  Synthetic oligonucleotide
gcccccagagacttgttgta